European Patent Application EP 4 257 703 A1, published October 11, 2023. Title: Method for selecting mesenchymal stem cell with improved self-maintenance and mesenchymal stem cells selected by thereof. Applicant: Samsung Life Public Welfare Foundation ENCELL CO., LTD. The sequence listing filed with the application follows.

SEQUENCE LISTING (12 sequences)

SEQ ID NO: 1 - RNA, 19 nt, Artificial
  siRNA of human AURKA
gagucauagcaugugugua

SEQ ID NO: 2 - RNA, 19 nt, Artificial
  siRNA of human AURKA
uacacacaugcuaugacuc

SEQ ID NO: 3 - RNA, 19 nt, Artificial
  siRNA of human AURKA
cugucauucgaagagaguu

SEQ ID NO: 4 - RNA, 19 nt, Artificial
  siRNA of human AURKA
aacucucuucgaaugacag

SEQ ID NO: 5 - RNA, 19 nt, Artificial
  siRNA of human AURKA
gugcaauaaccuuccuagu

SEQ ID NO: 6 - RNA, 19 nt, Artificial
  siRNA of human AURKA
acuaggaagguuauugcac

SEQ ID NO: 7 - RNA, 19 nt, Artificial
  siRNA of human DOCK2
cagaacaaaaucugcuuca

SEQ ID NO: 8 - RNA, 19 nt, Artificial
  siRNA of human DOCK2
ugaagcagauuuuguucug

SEQ ID NO: 9 - RNA, 18 nt, Artificial
  siRNA of human DOCK2
cugagaaugacuuccuac

SEQ ID NO: 10 - RNA, 19 nt, Artificial
  siRNA of human DOCK2
uguaggaagucauucucag

SEQ ID NO: 11 - RNA, 19 nt, Artificial
  siRNA of human DOCK2
cagaugagagcaaagacaa

SEQ ID NO: 12 - RNA, 19 nt, Artificial
  siRNA of human DOCK2
uugucuuugcucucaucug